European Patent Specification EP 4 087 860 B1, published November 22, 2023. Title: Compound and method for treatment of Alzheimer's disease. Applicant: AlphaBeta AB. The sequence listing filed with the application follows.

SEQUENCE LISTING (16 sequences)

SEQ ID NO: 1 - protein, 266 aa, Homo sapiens
MVKVTFNSALAQKEAKKDEPKSGEEALIIPPDAVAVDCKDPDDVVPVGQRRAWCWCMCFGLAFMLAGVILGGAYLYKYFALQPDDVYYCGIKYIKDDVILNEPSADAPAALYQTIEENIKIFEEEEVEFISVPVPEFADSDPANIVHDFNKKLTAYLDLNLDKCYVIPLNTSIVMPPRNLLELLINIKAGTYLPQSYLIHEHMVITDRIENIDHLGFFIYRLCHDKETYKLQRRETIKGIQKREASNCFAIRHFENKFAVETLICS

SEQ ID NO: 2 - protein, 270 aa, Artificial Sequence
  mutant
MGHHHHHHMSHTTPWTNPGLAENFMNSFMQGLSSMPGFTASQLDKMSTIAQSMVQSIQSLAAQGRTSPNDLQALNMAFASSMAEIAASEEGGGSLSTKTSSIASAMSNAFLQTTGVVNQPFINEITQLVSMFAQAGMNDVSAGNSLVPRGSQTIEENIKIFEEEEVEFISVPVPEFADSDPANIVHDFNKKLTAYLDLNLDKCYVIPLNTSIVMPPRNLLELLINIKAGTYLPQSYLIHEHMVITDRIENIDHLGFFIYELCHDKETYKL

SEQ ID NO: 3 - protein, 119 aa, Homo sapiens
QTIEENIKIFEEEEVEFISVPVPEFADSDPANIVHDFNKKLTAYLDLNLDKCYVIPLNTSIVMPPRNLLELLINIKAGTYLPQSYLIHEHMVITDRIENIDHLGFFIYRLCHDKETYKL

SEQ ID NO: 4 - protein, 119 aa, Artificial Sequence
  mutant
QTIEENIKIFEEEEVEFISVPVPEFADSDPANIVHDFNKKLTAYLDLNLDKCYVIPLNTSIVMPPRNLLELLINIKAGTYLPQSYLIHEHMVITDRIENIDHLGFFIYELCHDKETYKL

SEQ ID NO: 5 - protein, 89 aa, Homo sapiens
MVKVTFNSALAQKEAKKDEPKSGEEALIIPPDAVAVDCKDPDDVVPVGQRRAWCWCMCFGLAFMLAGVILGGAYLYKYFALQPDDVYYC

SEQ ID NO: 6 - protein, 23 aa, Homo sapiens
EASNCFAIRHFENKFAVETLICS

SEQ ID NO: 7 - protein, 95 aa, Homo sapiens
FADSDPANIVHDFNKKLTAYLDLNLDKCYVIPLNTSIVMPPRNLLELLINIKAGTYLPQSYLIHEHMVITDRIENIDHLGFFIYRLCHDKETYKL

SEQ ID NO: 8 - protein, 95 aa, Pan troglodytes; identical to SEQ ID NO: 7

SEQ ID NO: 9 - protein, 95 aa, Bos taurus
FADSDPANIVHDFNKKLTAYLDLNLDKCYVIPLNTSIVMPPKNLLELLINIKAGTYLPQSYLIHEHMVITDRIENIDHLGFYIYRLCHDKETYKL

SEQ ID NO: 10 - protein, 95 aa, Sus scrofa
FADSDPANIVHDFNKKLTAYLDLNLDKCYVIPLNTSIVMPPRNLLELLINIKAGTYLPQSYLIHEHMVITDRIENIDHLGFYIYRLCHDKETYKL

SEQ ID NO: 11 - protein, 95 aa, Mus musculus
FADSDPANIVHDFNKKLTAYLDLNLDKCYVIPLNTSIVMPPKNLLELLINIKAGTYLPQSYLIHEHMVITDRIENVDNLGFFIYRLCHDKETYKL

SEQ ID NO: 12 - protein, 95 aa, Rattus norvegicus
FADSDPANIVHDFNKKLTAYLDLNLDKCYVIPLNTSIVMPPRNLLELLINIKAGTYLPQSYLIHEHMVITDRIENVDHLGFFIYRLCHDKETYKL

SEQ ID NO: 13 - protein, 95 aa, Artificial Sequence
  mutant
FADSDPANIVHDFNKKLTAYLDLNLDKCYVIPLNTSIVMPPRNLLELLINIKAGTYLPQSYLIHEHMVITDRIENIDHLGFFIYELCHDKETYKL

SEQ ID NO: 14 - DNA, 44 bp, Homo sapiens
cacctgggtttctttatttatgaactgtgtcatgacaaggaaac

SEQ ID NO: 15 - DNA, 44 bp, Homo sapiens
gtttccttgtcatgacacagttcataaataaagaaacccaggtg

SEQ ID NO: 16 - DNA, 810 bp, Artificial Sequence
  mutant
atgggccatcatcatcatcatcatatgtcacacactacaccatggacaaacccaggactcgcagaaaacttcatgaacagtttcatgcaaggcctgagctcgatgccaggtttcacggcaagccaattggataagatgtcaaccatcgcacaatccatggtacagtcaatacaatccttggcggcacaaggcaggacatcaccgaatgacctgcaggcccttaacatggcttttgcatcttcgatggcagaaatcgcggcatccgaagaaggagggggaagcctttccaccaaaactagctctatagccagtgcaatgtccaacgcgtttctgcaaacaactggagtggtaaaccaaccgttcataaatgaaataactcagctcgttagcatgtttgctcaagcaggtatgaatgatgtcagtgctgggaattccctggtgccacgcggttctcagacaattgaagaaaatattaaaatctttgaagaagaagaagttgaatttatcagtgtgcctgtcccagagtttgcagatagtgatcctgccaacattgttcatgactttaacaagaaacttacagcctatttagatcttaacctggataagtgctatgtgatccctctgaacacttccattgttatgccacccagaaacctactggagttacttattaacatcaaggctggaacctatttgcctcagtcctatctgattcatgagcacatggttattactgatcgcattgaaaacattgatcacctgggtttctttatttatgaactgtgtcatgacaaggaaacttacaaactg